European Patent Application EP 4 112 057 A1, published January 4, 2023. Title: COMPOSITIONS AND METHODS OF USE OF ANTIBACTERIAL DRUG COMBINATIONS. Applicant: UNIVERSITY OF NOTRE DAME DU LAC. The sequence listing filed with the application follows.

SEQUENCE LISTING (8 sequences)

SEQ ID NO: 1 - DNA, 24 bp, Artificial Sequence
  SYNTHESIZED
cgtgccgaaatcaatgaaagacgc

SEQ ID NO: 2 - DNA, 24 bp, Artificial Sequence
  SYNTHESIZED
ggcaccttcagaaccaaatccacc

SEQ ID NO: 3 - DNA, 24 bp, Artificial Sequence
  SYNTHESIZED
tggaacgatgcctatctcatatgc

SEQ ID NO: 4 - DNA, 23 bp, Artificial Sequence
  SYNTHESIZED
caggaatgcagaaagaccaaagc

SEQ ID NO: 5 - DNA, 30 bp, Artificial Sequence
  SYNTHESIZED
tttatcagcaaccttatagtcttttggaac

SEQ ID NO: 6 - DNA, 20 bp, Artificial Sequence
  SYNTHESIZED
cctgctgctttcggcaagac

SEQ ID NO: 7 - DNA, 24 bp, Artificial Sequence
  SYNTHESIZED
cgatgtggatggagcgcatattag

SEQ ID NO: 8 - DNA, 23 bp, Artificial Sequence
  SYNTHESIZED
acaacggtggctgtgcaatatac